European Patent Application EP 4 628 105 A2, published October 8, 2025. Title: MULTISPECIFIC ANTIGEN-BINDING MOLECULE WITH IMPROVED INTERNALIZATION CHARACTERISTICS. Applicant: Genmab A/S. The sequence listing filed with the application follows.

SEQUENCE LISTING (12 sequences)

SEQ ID NO: 1 - protein, 120 aa, Homo sapiens
EVQLQQSGPELVKPGASVKMSCKASGYTFTSYVMHWVRQTPGQGLEWIGYITPYNDGTKYNEKFKGKATLTSDKSSSTAYMELSSLTSEDSAVYYCVGGDNYYYAMDYWGQGTSVTVSAA

SEQ ID NO: 2 - protein, 8 aa, Homo sapiens
GYTFTSYV

SEQ ID NO: 3 - protein, 8 aa, Homo sapiens
ITPYNDGT

SEQ ID NO: 4 - protein, 12 aa, Homo sapiens
VGGDNYYYAMDY

SEQ ID NO: 5 - protein, 114 aa, Homo sapiens
NIMVTQSPSSLAVSAGEKVTMSCKSSQSVLYSSNQKNYLAWYQQKPGQSPKLLIYWASTRVSGVPDRFTGSGSGTDFTLTISRVQAEDLAVYYCHQYFSSFTFGSGTKLEIKRT

SEQ ID NO: 6 - protein, 12 aa, Homo sapiens
QSVLYSSNQKNY

SEQ ID NO: 7 - skipped

SEQ ID NO: 8 - protein, 8 aa, Homo sapiens
HQYFSSFT

SEQ ID NO: 9 - protein, 12 aa, Homo sapiens
QSVLYSSHQKNY

SEQ ID NO: 10 - protein, 8 aa, Homo sapiens
IHPYNDGT

SEQ ID NO: 11 - protein, 8 aa, Homo sapiens
ITHYNDGT

SEQ ID NO: 12 - protein, 8 aa, Homo sapiens
ITPYHDGT